European Patent Application EP 4 644 531 A1, published November 5, 2025. Title: Probiotic Compositions for Preventing and Treating Cancer Treatment–related Diarrhea and Uses thereof. Applicant: SICHUAN ANAEROBIC BIOTECHNOLOGY CO., LTD. Application CN. The sequence listing filed with the application follows.

SEQUENCE LISTING (16 sequences)

SEQ ID NO: 1 - DNA, 20 bp, synthetic construct
  source 1..20: mol_type = other DNA
ctaaggccaaccgtgaaaag

SEQ ID NO: 2 - DNA, 20 bp, synthetic construct
  source 1..20: mol_type = other DNA
accagaggcatacagggaca

SEQ ID NO: 3 - DNA, 19 bp, synthetic construct
  source 1..19: mol_type = other DNA
ctgtagcccacgtcgtagc

SEQ ID NO: 4 - DNA, 18 bp, synthetic construct
  source 1..18: mol_type = other DNA
ttgagatccatgccgttg

SEQ ID NO: 5 - DNA, 19 bp, synthetic construct
  source 1..19: mol_type = other DNA
agttgacggaccccaaaag

SEQ ID NO: 6 - DNA, 20 bp, synthetic construct
  source 1..20: mol_type = other DNA
agctggatgctctcatcagg

SEQ ID NO: 7 - DNA, 20 bp, synthetic construct
  source 1..20: mol_type = other DNA
tgacgaccagaacatccaga

SEQ ID NO: 8 - DNA, 20 bp, synthetic construct
  source 1..20: mol_type = other DNA
aatcgccttgatctctccac

SEQ ID NO: 9 - DNA, 20 bp, synthetic construct
  source 1..20: mol_type = other DNA
gatcattccacgcagtctcc

SEQ ID NO: 10 - DNA, 20 bp, synthetic construct
  source 1..20: mol_type = other DNA
ggccccaggtttagacattc

SEQ ID NO: 11 - DNA, 22 bp, synthetic construct
  source 1..22: mol_type = other DNA
gcgatcatacccagagtctttc

SEQ ID NO: 12 - DNA, 20 bp, synthetic construct
  source 1..20: mol_type = other DNA
tgcctgaagtcatccacact

SEQ ID NO: 13 - DNA, 27 bp, synthetic construct
  source 1..27: mol_type = other DNA
ctacagggtttcatccaggatcgagca

SEQ ID NO: 14 - DNA, 21 bp, synthetic construct
  source 1..21: mol_type = other DNA
catgtcagctgccacccggaa

SEQ ID NO: 15 - DNA, 23 bp, synthetic construct
  source 1..23: mol_type = other DNA
tcaagaccatgctgctaattccc

SEQ ID NO: 16 - DNA, 19 bp, synthetic construct
  source 1..19: mol_type = other DNA
ggactcaccactttagcca